European Patent Application EP 4 249 589 A1, published September 27, 2023. Title: In vitro genetic disease model cell and method for producing the same. Applicant: Ricoh Company, Ltd. Application EP. The sequence listing filed with the application follows.

SEQUENCE LISTING (4 sequences)

SEQ ID NO: 1 - protein, 498 aa, Homo sapiens [sequence omitted]

SEQ ID NO: 2 - DNA, 1499 bp, Homo sapiens
  source 1..1499: mol_type = unassigned DNA
aaatggccgccgccgccgccgccgcgccgagcggaggaggaggaggaggcgaggaggagagactggaagaaaagtcagaagaccaggacctccagggcctcaaggacaaacccctcaagtttaaaaaggtgaagaaagataagaaagaagagaaagagggcaagcatgagcccgtgcagccatcagcccaccactctgctgagcccgcagaggcaggcaaagcagagacatcagaagggtcaggctccgccccggctgtgccggaagcttctgcctcccccaaacagcggcgctccatcatccgtgaccggggacccatgtatgatgaccccaccctgcctgaaggctggacacggaagcttaagcaaaggaaatctggccgctctgctgggaagtatgatgtgtatttgatcaatccccagggaaaagcctttcgctctaaagtggagttgattgcgtacttcgaaaaggtaggcgacacatccctggaccctaatgattttgacttcacggtaactgggagagggagcccctcccggcgagagcagaaaccacctaagaagcccaaatctcccaaagctccaggaactggcagaggccggggacgccccaaagggagcggcaccacgagacccaaggcggccacgtcagagggtgtgcaggtgaaaagggtcctggagaaaagtcctgggaagctccttgtcaagatgccttttcaaacttcgccagggggcaaggctgaggggggtggggccaccacatccacccaggtcatggtgatcaaacgccccggcaggaagcgaaaagctgaggccgaccctcaggccattcccaagaaacggggccgaaagccggggagtgtggtggcagccgctgccgccgaggccaaaaagaaagccgtgaaggagtcttctatccgatctgtgcaggagaccgtactccccatcaagaagcgcaagacccgggagacggtcagcatcgaggtcaaggaagtggtgaagcccctgctggtgtccaccctcggtgagaagagcgggaaaggactgaagacctgtaagagccctgggcggaaaagcaaggagagcagccccaaggggcgcagcagcagcgcctcctcaccccccaagaaggagcaccaccaccatcaccaccactcagagtccccaaaggcccccgtgccactgctcccacccctgcccccacctccacctgagcccgagagctccgaggaccccaccagcccccctgagccccaggacttgagcagcagcgtctgcaaagaggagaagatgcccagaggaggctcactggagagcgacggctgccccaaggagccagctaagactcagcccgcggttgccaccgccgccacggccgcagaaaagtacaaacaccgaggggagggagagcgcaaagacattgtttcatcctccatgccaaggccaaacagagaggagcctgtggacagccggacgcccgtgaccgagagagttagctga

SEQ ID NO: 3 - DNA, 41 bp, synthetic construct
  misc_feature 1..41: note = synthetic (shRNA)
  source 1..41: mol_type = other DNA
gggtagggctctgacaaagcttcccgattaactgaaataaa

SEQ ID NO: 4 - DNA, 41 bp, synthetic construct
  misc_feature 1..41: note = synthetic (shRNA)
  source 1..41: mol_type = other DNA
gaaacaccggcaacaagatgaagagcaccaactcgagttgg